European Patent Application EP 4 495 135 A1, published January 22, 2025. Title: PHARMACEUTICAL USE OF POLYPEPTIDE IN PREPARATION OF DRUGS FOR TREATING AND/OR PREVENTING DIABETES AND OBESITY AND RELATED DISEASES THEREOF. Applicant: GUANGDONG RAYNOVENT BIOTECH CO., LTD. Application EP. The sequence listing filed with the application follows.

SEQUENCE LISTING (11 sequences)

SEQ ID NO: 1 - protein, 39 aa, synthetic construct
  SITE 13: note = Aib
  SITE 2: note = Aib
  SITE 39: note = (S)-2-amino-3-hydroxypropionic acid or (S)-2-amino-3-hydroxypropanamide
YXEGTFTSDYSIXLDKIAQKAFVKWLIAGGPSSGAPPPX

SEQ ID NO: 2 - protein, 39 aa, synthetic construct
  SITE 2: note = Aib
  SITE 39: note = (S)-2-amino-3-hydroxypropionic acid or (S)-2-amino-3-hydroxypropanamide
  SITE 13: note = Aib
YXEGTFTSDYSIXLDKKAQKAFVKWLIAGGPSSGAPPPX

SEQ ID NO: 3 - protein, 39 aa, synthetic construct
  SITE 13: note = Aib
  SITE 2: note = Aib
  MOD_RES 39: note = AMIDATION
YXEGTFTSDYSIXLDKIAQKAFVKWLIAGGPSSGAPPPS

SEQ ID NO: 4 - protein, 39 aa, synthetic construct
  SITE 2: note = Aib
  SITE 13: note = Aib
  MOD_RES 39: note = AMIDATION
YXEGTFTSDYSIXLDKIAQKEFVKWLIAGGPSSGAPPPS

SEQ ID NO: 5 - protein, 39 aa, synthetic construct
  SITE 13: note = Aib
  MOD_RES 39: note = AMIDATION
  SITE 2: note = Aib
YXEGTFTSDYSIXLDKIAQKAFIKWLIAGGPSSGAPPPS

SEQ ID NO: 6 - protein, 39 aa, synthetic construct
  SITE 13: note = Aib
  SITE 2: note = Aib
  MOD_RES 39: note = AMIDATION
YXEGTFTSDYSIXLDKIAQKAFVKWLLAGGPSSGAPPPS

SEQ ID NO: 7 - protein, 39 aa, synthetic construct
  SITE 13: note = Aib
  SITE 2: note = Aib
  MOD_RES 39: note = AMIDATION
YXEGTFTSDYSIXLDKKAQKAFVEWLIAGGPSSGAPPPS

SEQ ID NO: 8 - protein, 39 aa, synthetic construct
  SITE 13: note = Aib
  SITE 2: note = Aib
  MOD_RES 39: note = AMIDATION
YXEGTFTSDYSIXLDKKAQKAFVQWLIAGGPSSGAPPPS

SEQ ID NO: 9 - protein, 39 aa, synthetic construct
  SITE 13: note = Aib
  SITE 2: note = Aib
  MOD_RES 39: note = AMIDATION
YXEGTFTSDYSIXLDKKAQKAFVAWLIAGGPSSGAPPPS

SEQ ID NO: 10 - protein, 39 aa, synthetic construct
  SITE 13: note = Aib
  SITE 2: note = Aib
  MOD_RES 39: note = AMIDATION
YXEGTFTSDYSIXLDKKAQKAFVIWLIAGGPSSGAPPPS

SEQ ID NO: 11 - protein, 39 aa, synthetic construct
  SITE 13: note = Aib
  SITE 2: note = Aib
  MOD_RES 39: note = AMIDATION
YXEGTFTSDYSIXLDKKAQKEFVEWLIAGGPSSGAPPPS